European Patent Application EP 4 279 140 A2, published November 22, 2023. Title: HUMAN ANTIBODIES AGAINST TISSUE FACTOR. Applicant: Genmab. The sequence listing filed with the application follows.

SEQUENCE LISTING (112 sequences)

SEQ ID NO: 1 - protein, 126 aa, Homo sapiens
EVQLVQSGAEVKKPGESLKISCKGSGYSFTSYWIGWVRQMPGKGLEWMGIIYPGDSDTRYSPSFQGQVTISADKSISTAYLQWSSLKASDTAMYYCARIHRGAGYSSSWPGAFDIWGQGTMVTVSS

SEQ ID NO: 2 - protein, 8 aa, Homo sapiens
GYSFTSYW

SEQ ID NO: 3 - protein, 8 aa, Homo sapiens
IYPGDSDT

SEQ ID NO: 4 - protein, 19 aa, Homo sapiens
ARIHRGAGYSSSWPGAFDI

SEQ ID NO: 5 - protein, 119 aa, Homo sapiens
QVQLVESGGGVVQPGRSLRLSCVASGFTVSNDGMHWVRQAPGKGLEWVALIWYDGVNKNYADSVKGRFTISRDKSKNTLYLQMNSLRAEDTAVYYCARRPGTFYGLDVWGQGTTVTVSS

SEQ ID NO: 6 - protein, 8 aa, Homo sapiens
GFTVSNDG

SEQ ID NO: 7 - protein, 8 aa, Homo sapiens
IWYDGVNK

SEQ ID NO: 8 - protein, 12 aa, Homo sapiens
ARRPGTFYGLDV

SEQ ID NO: 9 - protein, 118 aa, Homo sapiens
EVQLLESGGGLVQPGGSLRLSCAASGFTFSNYAMSWVRQAPGKGLEWVSSISGSGDYTYYTDSVKGRFTISRDNSKNTLYLQMNSLRAEDTAVYYCARSPWGYYLDSWGQGTLVTVSS

SEQ ID NO: 10 - protein, 8 aa, Homo sapiens
GFTFSNYA

SEQ ID NO: 11 - protein, 8 aa, Homo sapiens
ISGSGDYT

SEQ ID NO: 12 - protein, 11 aa, Homo sapiens
ARSPWGYYLDS

SEQ ID NO: 13 - protein, 120 aa, Homo sapiens
EVQLLESGGGLVQPGGSLRLSCAASGFTFSSYAMSWVRQAPGKGLEWVSAISGSGDSTNYADSVKGRFTISRDNSKNTLYLQMNSLRAEDTAVYYCAKDGYFLLWYFDLWGRGTLVTVSS

SEQ ID NO: 14 - protein, 8 aa, Homo sapiens
GFTFSSYA

SEQ ID NO: 15 - protein, 8 aa, Homo sapiens
ISGSGDST

SEQ ID NO: 16 - protein, 13 aa, Homo sapiens
AKDGYFLLWYFDL

SEQ ID NO: 17 - protein, 118 aa, Homo sapiens
EVQLLESGGGLVQPGGSLRLSCAASGFTFSSYGMSWVRQAPGKGLEWVSVISGSGGTTYYADSVKGRFTISRDNSKNTLYLQMNSLRAEDTAVYYCAKAPWTYYFDYWGQGTLVTVSS

SEQ ID NO: 18 - protein, 8 aa, Homo sapiens
GFTFSSYG

SEQ ID NO: 19 - protein, 8 aa, Homo sapiens
ISGSGGTT

SEQ ID NO: 20 - protein, 11 aa, Homo sapiens
AKAPWTYYFDY

SEQ ID NO: 21 - protein, 118 aa, Homo sapiens
EVQLLESGGGLVQPGGSLRLSCAASGFTFNNYAMSWVRQAPGKGLEWVSSISGSGGRTYYADSVKGRFTISRDNSKNTLFLQMNSLRAEDTAVYYCAKTPWGYYFDYWGQGTLVTVSS

SEQ ID NO: 22 - protein, 8 aa, Homo sapiens
GFTFNNYA

SEQ ID NO: 23 - protein, 8 aa, Homo sapiens
ISGSGGRT

SEQ ID NO: 24 - protein, 11 aa, Homo sapiens
AKTPWGYYFDY

SEQ ID NO: 25 - protein, 118 aa, Homo sapiens
EVQLLESGGGLVQPGGSLRLSCAASGFTFSNYAMSWVRQAPAKGLDWVSGISGSGVTTYYADSVKGRFTISRDNSKDTLYLQMNSLRAEDTAVYFCAKTPWGYYFDYWGQGILVAVSS

SEQ ID NO: 26 - protein, 8 aa, Homo sapiens
GFTFSNYA

SEQ ID NO: 27 - protein, 8 aa, Homo sapiens
ISGSGVTT

SEQ ID NO: 28 - protein, 11 aa, Homo sapiens
AKTPWGYYFDY

SEQ ID NO: 29 - protein, 118 aa, Homo sapiens
QVQLVQSGAEVKKPGSSVKVSCKAPRGTFSYYTISWVRQAPGQGLEWMGRIIPILGVANYAQKFQGRVTITADKSTSTAYMELSSLRSEDTAVYYCAREGDRRYFDYWGQGTLVTVSS

SEQ ID NO: 30 - protein, 8 aa, Homo sapiens
RGTFSYYT

SEQ ID NO: 31 - protein, 8 aa, Homo sapiens
IIPILGVA

SEQ ID NO: 32 - protein, 11 aa, Homo sapiens
AREGDRRYFDY

SEQ ID NO: 33 - protein, 120 aa, Homo sapiens
QVQLVESGGGVVQPGRSLRLSCAASGFTFSRYAMHWVRQAPGKGLEWVAVISNDGYNDYYADSVKGRFTVSRDNSKNTLYLQMNSLRAEDTAVYYCARDGQLGRGYFDYWGQGTLVTVSS

SEQ ID NO: 34 - protein, 8 aa, Homo sapiens
GFTFSRYA

SEQ ID NO: 35 - protein, 8 aa, Homo sapiens
ISNDGYND

SEQ ID NO: 36 - protein, 13 aa, Homo sapiens
ARDGQLGRGYFDY

SEQ ID NO: 37 - protein, 120 aa, Homo sapiens
QVQLVESGGGVVQPGRSLRLSCPASGFTFSIYAMHWVRQAPGKGLEWVAVVSNDGYNKYYADSVKGRFTISRDNSKDTLYLQMNSLRAEDTAVYYCARDGQLGRGYFDYWGQGTLVTVSS

SEQ ID NO: 38 - protein, 8 aa, Homo sapiens
GFTFSIYA

SEQ ID NO: 39 - protein, 8 aa, Homo sapiens
VSNDGYNK

SEQ ID NO: 40 - protein, 13 aa, Homo sapiens
ARDGQLGRGYFDY

SEQ ID NO: 41 - protein, 118 aa, Homo sapiens
QVQLVESGGGVVQPGRSLRLSCAASGFTFSDYAMHWVRQAPGKGLEWVAVIPYDGDNKYYADSVKGRFTISRDNSKNTLYLQMNSLRAEDTAVYYCAREDWGLEVDYWGQGALVTVSS

SEQ ID NO: 42 - protein, 8 aa, Homo sapiens
GFTFSDYA

SEQ ID NO: 43 - protein, 8 aa, Homo sapiens
IPYDGDNK

SEQ ID NO: 44 - protein, 11 aa, Homo sapiens
AREDWGLEVDY

SEQ ID NO: 45 - protein, 121 aa, Homo sapiens
EVQLVQSGAEVKKPGESLKISCKGSGYSFTSCWIGWVRQMPGKGLEWMGIIYPGDSDTRYSPSFQGQVTISADKSISTAYLQWSSLKASDTAMYYCARHKLGMDHDAFDIWGQGTMVTVSS

SEQ ID NO: 46 - protein, 8 aa, Homo sapiens
GYSFTSCW

SEQ ID NO: 47 - protein, 8 aa, Homo sapiens
IYPGDSDT

SEQ ID NO: 48 - protein, 14 aa, Homo sapiens
ARHKLGMDHDAFDI

SEQ ID NO: 49 - protein, 118 aa, Homo sapiens
QVQLVQSGAEVRKPGSSVKVSCKASGGSFNNYPIFWVRQAPGQGFEWMGRIIPILGITAYAQKFQGRVTITADKSTSTAYMELNSLRSEDTAVYYCAGGDDLDAFDIWGQGTMVSVSS

SEQ ID NO: 50 - protein, 8 aa, Homo sapiens
GGSFNNYP

SEQ ID NO: 51 - protein, 8 aa, Homo sapiens
IIPILGIT

SEQ ID NO: 52 - protein, 11 aa, Homo sapiens
AGGDDLDAFDI

SEQ ID NO: 53 - protein, 120 aa, Homo sapiens
QVQLVESGGGVVQPGRSLRLSCAGSGFTFNRYAMYWVRQAPGKGLDWVAVISNDGINKYYADSVKGRFTISRDNSKNTLYLQMNSLRAEDTAVYYCARDHTMVRGAFDYWGQGTLVTVSS

SEQ ID NO: 54 - protein, 8 aa, Homo sapiens
GFTFNRYA

SEQ ID NO: 55 - protein, 8 aa, Homo sapiens
ISNDGINK

SEQ ID NO: 56 - protein, 13 aa, Homo sapiens
ARDHTMVRGAFDY

SEQ ID NO: 57 - protein, 107 aa, Homo sapiens
DIQMTQSPSSLSASVGDRVTITCRASQGISRWLAWYQQKPEKAPKSLIYAASSLQSGVPSRFSGSGSGTDFTLTISSLQPEDFATYYCQQYDSDPITFGQGTRLEIK

SEQ ID NO: 58 - protein, 6 aa, Homo sapiens
QGISRW

SEQ ID NO: 59 - skipped

SEQ ID NO: 60 - protein, 9 aa, Homo sapiens
QQYDSDPIT

SEQ ID NO: 61 - protein, 107 aa, Homo sapiens
EIVLTQSPGTLSLSPGERATLSCRASQSVSSSYLAWYQQKPGQAPRLLIYGASSRATGIPDRFSGSGSGTDFTLTISRLEPEDFAVYYCQQYGSSLTFGGGTKVEIK

SEQ ID NO: 62 - protein, 7 aa, Homo sapiens
QSVSSSY

SEQ ID NO: 63 - skipped

SEQ ID NO: 64 - protein, 8 aa, Homo sapiens
QQYGSSLT

SEQ ID NO: 65 - protein, 107 aa, Homo sapiens
DIQMTQSPPSLSASAGDRVTITCRASQGISSRLAWYQQKPEKAPKSLIYAASSLQSGVPSRFSGSGSGTDFTLTISSLQPEDFATYYCQQYNSYPYTFGQGTKLEIK

SEQ ID NO: 66 - protein, 6 aa, Homo sapiens
QGISSR

SEQ ID NO: 67 - skipped

SEQ ID NO: 68 - protein, 9 aa, Homo sapiens
QQYNSYPYT

SEQ ID NO: 69 - protein, 108 aa, Homo sapiens
EIVLTQSPGTLSLSPGERATLSCRASQSVRSSYLAWYQQKPGQAPRLLIYGASSRATGIPDRFSGSGSGTDFTLTISRLEPEDFAVYYCQQYGSSPRTFGQGTKVEIK

SEQ ID NO: 70 - protein, 7 aa, Homo sapiens
QSVRSSY

SEQ ID NO: 71 - skipped

SEQ ID NO: 72 - protein, 9 aa, Homo sapiens
QQYGSSPRT

SEQ ID NO: 73 - protein, 108 aa, Homo sapiens
EIVLTQSPGTLSLSPGERATLSCRASQSVGSSSLAWYQQKPGQAPRLLIYGASSRATGIPDRFSGSGSGTDFTLTISRLEPEDFAVYYCQQYGSSPRTFGQGTKVEIK

SEQ ID NO: 74 - protein, 7 aa, Homo sapiens
QSVGSSS

SEQ ID NO: 75 - skipped

SEQ ID NO: 76 - protein, 9 aa, Homo sapiens
QQYGSSPRT

SEQ ID NO: 77 - protein, 107 aa, Homo sapiens
DIQMTQSPSSLSASVGDRVTITCRASQGISSRLAWYQQKPEKAPKSLIYAASSLQSGVPSRFSGSGSGTDFTLTISSLQPEDFATYYCQQYNSYPYTFGQGTKLEIK

SEQ ID NO: 78 - protein, 6 aa, Homo sapiens
QGISSR

SEQ ID NO: 79 - skipped

SEQ ID NO: 80 - protein, 9 aa, Homo sapiens
QQYNSYPYT

SEQ ID NO: 81 - protein, 108 aa, Homo sapiens
DIQMTQSPSSLSASVGDRVTITCRASQGISSWLAWYQQKPEKAPKSLIYAASSLQSGVPSRFSGSGSGTDFTLTISSLQPEDFATYYCQQYNSYPLYTFGQGTKLEIK

SEQ ID NO: 82 - protein, 6 aa, Homo sapiens
QGISSW

SEQ ID NO: 83 - skipped

SEQ ID NO: 84 - protein, 10 aa, Homo sapiens
QQYNSYPLYT

SEQ ID NO: 85 - protein, 107 aa, Homo sapiens
AIQLTQSPSSLSASVGDRVTITCRASQDISSALAWYQQKPGKAPKLLIYDASILESGVPSRFSGSGSGTDFTLTISSLQPEDFATYYCQQFNSYPLTFGGGTKVEIK

SEQ ID NO: 86 - protein, 6 aa, Homo sapiens
QDISSA

SEQ ID NO: 87 - skipped

SEQ ID NO: 88 - protein, 9 aa, Homo sapiens
QQFNSYPLT

SEQ ID NO: 89 - protein, 107 aa, Homo sapiens
EIVLTQSPATLSLSPGERATLSCRASQSVSSYLAWYQQKPGQAPRLLIYDASNRATGIPARFSGSGSGTDFTLTISSLEPEDFAVYYCQQRSNWPLTFGGGTKVEIK

SEQ ID NO: 90 - protein, 6 aa, Homo sapiens
QSVSSY

SEQ ID NO: 91 - skipped

SEQ ID NO: 92 - protein, 9 aa, Homo sapiens
QQRSNWPLT

SEQ ID NO: 93 - protein, 107 aa, Homo sapiens
EIVLTQSPATLSLSPGERAILSCRASQSVSSYLAWYQQKPGQAPRLLIYDASNRATGIPARFSGSGSGTDFTLTISSLEPEDFAVYYCQQRSNWPLTFGGGTKVEIK

SEQ ID NO: 94 - protein, 6 aa, Homo sapiens
QSVSSY

SEQ ID NO: 95 - skipped

SEQ ID NO: 96 - protein, 9 aa, Homo sapiens
QQRSNWPLT

SEQ ID NO: 97 - protein, 107 aa, Homo sapiens
AIQLTQSPSSLSASVGDRVTITCRASQGINSALAWYQQKPGKAPKLLIYDASSLESGVPSRFSGSGSGTDFTLTISSLQPEDFATYYCQQFNSYPLTFGGGTKVEIK

SEQ ID NO: 98 - protein, 6 aa, Homo sapiens
QGINSA

SEQ ID NO: 99 - skipped

SEQ ID NO: 100 - protein, 9 aa, Homo sapiens
QQFNSYPLT

SEQ ID NO: 101 - protein, 107 aa, Homo sapiens
DIQMTQSPSSLSASVGDRVTITCRASQGISSWLAWYQQKPEKAPKSLIYAASSLQSGVPSRFSGSGSGTDFTLTISSLQPEDFATYYCQQYNSYPPTFGQGTTVEVK

SEQ ID NO: 102 - protein, 6 aa, Homo sapiens
QGISSW

SEQ ID NO: 103 - skipped

SEQ ID NO: 104 - protein, 9 aa, Homo sapiens
QQYNSYPPT

SEQ ID NO: 105 - protein, 107 aa, Homo sapiens
DIQMTQSPSSLSASVGDRVTITCRASQGISSWLAWYQQKPEKAPKSLIYAASSLQSGVPSRFSGSGSGTDFTLTISSLQPEDFATYYCQQYNSYPYTFGQGTKLEIK

SEQ ID NO: 106 - protein, 6 aa, Homo sapiens
QGISSW

SEQ ID NO: 107 - skipped

SEQ ID NO: 108 - protein, 9 aa, Homo sapiens
QQYNSYPYT

SEQ ID NO: 109 - protein, 107 aa, Homo sapiens; identical to SEQ ID NO: 89

SEQ ID NO: 110 - protein, 6 aa, Homo sapiens
QSVSSY

SEQ ID NO: 111 - skipped

SEQ ID NO: 112 - protein, 9 aa, Homo sapiens
QQRSNWPLT